European Patent Application EP 4 176 872 A1, published May 10, 2023. Title: METHOD FOR CONTROLLING OBESITY BY REGULATING ACTIVITY OF TREK1. Applicant: KOREA INSTITUTE OF SCIENCE AND TECHNOLOGY. The sequence listing filed with the application follows.

SEQUENCE LISTING (1 sequence)

SEQ ID NO: 1 - DNA, 21 bp, synthetic construct
  source 1..21: mol_type = other DNA
gcgtggagatctacgacaagt